European Patent Specification EP 4 366 749 B1, published August 13, 2025. Title: Corynebacterium strains for use in the prevention of a viral infection. Applicant: Semmelweis Egyetem. The sequence listing filed with the application follows.

SEQUENCE LISTING (6 sequences)

SEQ ID NO: 1 - DNA, 24 bp, synthetic construct
  source 1..24: mol_type = other DNA
gggatcagagatcggaagaagaaa

SEQ ID NO: 2 - DNA, 23 bp, synthetic construct
  source 1..23: mol_type = other DNA
aggaggtctgaacatcatcagtg

SEQ ID NO: 3 - DNA, 21 bp, synthetic construct
  source 1..21: mol_type = other DNA
aatcggtgtgttcgcctctac

SEQ ID NO: 4 - DNA, 21 bp, synthetic construct
  source 1..21: mol_type = other DNA
cgtagttctcgttccagtcgt

SEQ ID NO: 5 - DNA, 22 bp, synthetic construct
  source 1..22: mol_type = other DNA
ctactggcgctggcaaggctgt

SEQ ID NO: 6 - DNA, 24 bp, synthetic construct
  source 1..24: mol_type = other DNA
gccatgaggtccaccaccctgctg